European Patent Application EP 4 186 514 A1, published May 31, 2023. Title: PHARMACEUTICAL COMPOSITION FOR PREVENTING OR TREATING CHOLANGITIS OR LIVER DISEASE CAUSED BY CHOLANGITIS COMPRISING ADENOSINE DERIVATIVE. Applicant: Future Medicine Co., Ltd. The sequence listing filed with the application follows.

SEQUENCE LISTING (8 sequences)

SEQ ID NO: 1 - DNA, 20 bp, Acta2 (NM_007392.3) F
tatgctaacaacgtcctgtc

SEQ ID NO: 2 - DNA, 20 bp, Acta2 (NM_007392.3) R
agacagagtacttgcgttct

SEQ ID NO: 3 - DNA, 20 bp, Col1a1 (NM_007742.4) F
gaacctaaccatctggcatc

SEQ ID NO: 4 - DNA, 20 bp, Col1a1 (NM_007742.4) R
aatagaacggtctctcccac

SEQ ID NO: 5 - DNA, 20 bp, Timp1 (NM_001044384.1) F
agacacaccagagcagatac

SEQ ID NO: 6 - DNA, 20 bp, Timp1 (NM_001044384.1) R
cgctggtataaggtggtctc

SEQ ID NO: 7 - DNA, 19 bp, Gapdh (NM_001289726.1) F
tgcaccaccaactgcttag

SEQ ID NO: 8 - DNA, 19 bp, Gapdh (NM_001289726.1) R
ggatgcagggatgatgttc